European Patent Application EP 4 324 924 A1, published February 21, 2024. Title: Novel promoter and use thereof. Applicant: CJ CheilJedang Corporation. The sequence listing filed with the application follows.

SEQUENCE LISTING (28 sequences)

SEQ ID NO: 1 - DNA, 330 bp, Corynebacterium glutamicum
attctttgtggtcatatctgtgcgacactgccataattgaacgtgagcatttaccagcctaaatgcccgcagtgagttaagtctcaaagcaagaagttgctctttagggcatccgtagtttaaaactattaaccgttaggtatgacaagccggttgatgtgaacgcagtttttaaaagtttcaggatcagatttttcacaggcattttgctccagcaaacgcctaggatgtacatggtgccctcaatgggaaccaccaacatcactaaatggcccaggtacacactttaaaatcgtgcgcgcatgcagccgagatgggaacgaggaaatc

SEQ ID NO: 2 - DNA, 330 bp, Artificial Sequence
  Pm3gdh
attctttgtggtcatatctgtgcgactgtggtatacttgaacgtgagcatttaccagcctaaatgcccgcagtgagttaagtctcaaagcaagaagttgctctttagggcatccgtagtttaaaactattaaccgttaggtatgacaagccggttgatgtgaacgcagtttttaaaagtttcaggatcagatttttcacaggcattttgctccagcaaacgcctaggatgtacatggtgccctcaatgggaaccaccaacatcactaaatggcccaggtacacactttaaaatcgtgcgcgcatgcagccgagatgggaacgaggaaatc

SEQ ID NO: 3 - DNA, 330 bp, Artificial Sequence
  Pm16gdh
attctttgtggtcatatctgtgcgactgtggtatacttgaacgtgagcatttaccagcctaaatgtccgcagtgagttaagtctcaaagcaagaagttgctctttagggcatccgtagtttaaaactattaaccgttaggtatgacaagccggttgatgtgaacgcagtttttaaaagtttcaggatcagatttttcacaggcattttgctccagcaaacgcctaggatgtacatggtgccctcaatgggaaccaccaacgtcactaaatggcccaggtacacactttaaaatcgtgcgcgcatgcagccgagatgggaacgaggaaatc

SEQ ID NO: 4 - DNA, 330 bp, Artificial Sequence
  Pm78gdh
attctttgtggtcatatctgtgcgactgtggtatacttgaacgtgagcatttaccagcctaaatgtccgcagtgagttaagtctcaaagcaagaagttgctctttagggcatccgtagtttaaaactattaaccgttaggtatgacaagccggttgatgtgaacgcagtttttaaaagtttcaggatcagatttttcacaggcattttgctccagcaaacgcctaggatgtacatggtgccctcaatgggaaccaccaacatcactaaatggcccaggtacacactttaaaatcgtgcgcgcatgcagccgagatgggaacgaggaaatc

SEQ ID NO: 5 - DNA, 39 bp, Artificial Sequence
  Pgdhm primer
ctctagaactagtggatccattctttgtggtcatatctg

SEQ ID NO: 6 - DNA, 40 bp, Artificial Sequence
  Pgdhm primer
agttcttctcctttactcatgatttcctcgttcccatctc

SEQ ID NO: 7 - DNA, 40 bp, Artificial Sequence
  GFP primer
gagatgggaacgaggaaatcatgagtaaaggagaagaact

SEQ ID NO: 8 - DNA, 37 bp, Artificial Sequence
  GFP primer
cccccctcgaggtcgacttatttgtagagctcatcca

SEQ ID NO: 9 - DNA, 20 bp, Artificial Sequence
  Pgdhm primer
attctttgtggtcatatctg

SEQ ID NO: 10 - DNA, 20 bp, Artificial Sequence
  Pgdhm primer
gatttcctcgttcccatctc

SEQ ID NO: 11 - DNA, 38 bp, Artificial Sequence
  pDZ-Pm3, 4, 6_gdh primer
gtgaattcgagctcggtaccccgtcggtgggggagttg

SEQ ID NO: 12 - DNA, 36 bp, Artificial Sequence
  pDZ-Pm3, 4, 6_gdh primer
gatatgaccacaaagaattaaaattgtttgaaaatt

SEQ ID NO: 13 - DNA, 36 bp, Artificial Sequence
  pDZ-Pm3, 4, 6_gdh primer
aattttcaaacaattttaattctttgtggtcatatc

SEQ ID NO: 14 - DNA, 38 bp, Artificial Sequence
  pDZ-Pm3, 4, 6_gdh primer
cctgctcatcaactgtcatgatttcctcgttcccatct

SEQ ID NO: 15 - DNA, 38 bp, Artificial Sequence
  pDZ-Pm3, 4, 6_gdh primer
agatgggaacgaggaaatcatgacagttgatgagcagg

SEQ ID NO: 16 - DNA, 39 bp, Artificial Sequence
  pDZ-Pm3, 4, 6_gdh primer
ggtcgactctagaggatcccccaactccgatgtcacctg

SEQ ID NO: 17 - DNA, 41 bp, Artificial Sequence
  lysC(L377K) primer
gtgaattcgagctcggtaccctccaagattttggtgctgcg

SEQ ID NO: 18 - DNA, 40 bp, Artificial Sequence
  lysC(L377K) primer
atctcagaggtggaaatcttttcgatgttcacgttgacat

SEQ ID NO: 19 - DNA, 40 bp, Artificial Sequence
  lysC(L377K) primer
atgtcaacgtgaacatcgaaaagatttccacctctgagat

SEQ ID NO: 20 - DNA, 41 bp, Artificial Sequence
  lysC(L377K) primer
ggtcgactctagaggatccccgttcacctcagagacgatta

SEQ ID NO: 21 - DNA, 41 bp, Artificial Sequence
  hom(R398Q) primer
gtgaattcgagctcggtaccctttccacacccgtgttaccg

SEQ ID NO: 22 - DNA, 40 bp, Artificial Sequence
  hom(R398Q) primer
atcatcgcgctcttcctgttggattgtacgcagggagatt

SEQ ID NO: 23 - DNA, 40 bp, Artificial Sequence
  hom(R398Q) primer
aatctccctgcgtacaatccaacaggaagagcgcgatgat

SEQ ID NO: 24 - DNA, 41 bp, Artificial Sequence
  hom(R398Q) primer
ggtcgactctagaggatccccaaccattagctgcagcaaca

SEQ ID NO: 25 - DNA, 20 bp, Artificial Sequence
  lysC(L377K) primer
tcctaatgcacagaagctgg

SEQ ID NO: 26 - DNA, 20 bp, Artificial Sequence
  lysC(L377K) primer
gtggtgcagttagggttcgc

SEQ ID NO: 27 - DNA, 20 bp, Artificial Sequence
  hom(R398Q) primer
atccaactgcagacgtcgaa

SEQ ID NO: 28 - DNA, 20 bp, Artificial Sequence
  hom(R398Q) primer
atctgggtggccttcaaagg